European Patent Specification EP 3 502 250 B1, published April 24, 2024. Title: GENE-MODIFIED NON-HUMAN ANIMALS EXPRESSING A HUMAN GPC3 POLYPEPTIDE. Applicant: CHUGAI SEIYAKU KABUSHIKI KAISHA. The sequence listing filed with the application follows.

SEQUENCE LISTING (74 sequences)

SEQ ID NO: 1 - protein, 580 aa, Homo sapiens
MAGTVRTACLVVAMLLSLDFPGQAQPPPPPPDATCHQVRSFFQRLQPGLKWVPETPVPGSDLQVCLPKGPTCCSRKMEEKYQLTARLNMEQLLQSASMELKFLIIQNAAVFQEAFEIVVRHAKNYTNAMFKNNYPSLTPQAFEFVGEFFTDVSLYILGSDINVDDMVNELFDSLFPVIYTQLMNPGLPDSALDINECLRGARRDLKVFGNFPKLIMTQVSKSLQVTRIFLQALNLGIEVINTTDHLKFSKDCGRMLTRMWYCSYCQGLMMVKPCGGYCNVVMQGCMAGVVEIDKYWREYILSLEELVNGMYRIYDMENVLLGLFSTIHDSIQYVQKNAGKLTTTIGKLCAHSQQRQYRSAYYPEDLFIDKKVLKVAHVEHEETLSSRRRELIQKLKSFISFYSALPGYICSHSPVAENDTLCWNGQELVERYSQKAARNGMKNQFNLHELKMKGPEPVVSQIIDKLKHINQLLRTMSMPKGRVLDKNLDEEGFESGDCGDDEDECIGGSGDGMIKVKNQLRFLAELAYDLDVDDAPGNSQQATPKDNEISTFHNLGNVHSPLKLLTSMAISVVCFFFLVH

SEQ ID NO: 2 - protein, 580 aa, Macaca fascicularis
MAGTVRTACLVVAMLLSLDFPGQAQPPPPPPDATCHQVRSFFQRLQPGLKWVPETPVPGSDLQVCLPKGPTCCSRKMEEKYQLTARLNMEQLLQSASMELKFLIIQNAAVFQEAFEIVVRHAKNYTNAMFKNNYPSLTPQAFEFVGEFFTDVSLYILGSDINVDDMVNELFDSLFPVIYTQLMNPGLPDSALDINECLRGARRDLKVFGNFPKLIMTQVSKSLQVTRIFLQALNLGIEVINTTDHLKFSKDCGRMLTRMWYCSYCQGLMMVKPCGGYCNVVMQGCMAGVVEIDKYWREYILSLEELVNGMYRIYDMENVLLGLFSTIHDSIQYVQKNAGKLTTTIGKLCAHSQQRQYRSAYYPEDLFIDKKVLKVAHVEHEETLSSRRRELIQKLKSFISFYSALPGYICSHSPVAENDTLCWNGQELVERYSQKAARNGMKNQFNLHELKMKGPEPVVSQIIDKLKHINQLLRTMSVPKGRVLDKNLDEEGFESGDCGDDEDECIGGSGDGMMKVKNQLRFLAELAYDLDVDDVPGNNQQATPKDNEISTFHNLGNVHSPLKLLTSMAISVVCFFFLVH

SEQ ID NO: 3 - protein, 579 aa, Mus musculus
MAGTVRTACLLVAMLLGLGCLGQAQPPPPPDATCHQVRSFFQRLQPGLKWVPETPVPGSDLQVCLPKGPTCCSRKMEEKYQLTARLNMEQLLQSASMELKFLIIQNAAVFQEAFEIVVRHAKNYTNAMFKNNYPSLTPQAFEFVGEFFTDVSLYILGSDINVDDMVNELFDSLFPVIYTQMMNPGLPESVLDINECLRGARRDLKVFGSFPKLIMTQVSKSLQVTRIFLQALNLGIEVINTTDHLKFSKDCGRMLTRMWYCSYCQGLMMVKPCGGYCNVVMQGCMAGVVEIDKYWREYILSLEELVNGMYRIYDMENVLLGLFSTIHDSIQYVQKNGGKLTTTIGKLCAHSQQRQYRSAYYPEDLFIDKKILKVAHVEHEETLSSRRRELIQKLKSFINFYSALPGYICSHSPVAENDTLCWNGQELVERYSQKAARNGMKNQFNLHELKMKGPEPVVSQIIDKLKHINQLLRTMSVPKGKVLDKSLDEEGLESGDCGDDEDECIGSSGDGMVKVKNQLRFLAELAYDLDVDDAPGNKQHGNQKDNEITTSHSVGNMPSPLKILISVAIYVACFFFLVH

SEQ ID NO: 4 - DNA, 2329 bp, Homo sapiens
agccccgccctgccccgcgccgccaagcggttcccgccctcgcccagcgcccaggtagctgcgaggaaacttttgcagcggctgggtagcagcacgtctcttgctcctcagggccactgccaggcttgccgagtcctgggactgctctcgctccggctgccactctcccgcgctctcctagctccctgcgaagcaggatggccgggaccgtgcgcaccgcgtgcttggtggtggcgatgctgctcagcttggacttcccgggacaggcgcagcccccgccgccgccgccggacgccacctgtcaccaagtccgctccttcttccagagactgcagcccggactcaagtgggtgccagaaactcccgtgccaggatcagatttgcaagtatgtctccctaagggcccaacatgctgctcaagaaagatggaagaaaaataccaactaacagcacgattgaacatggaacagctgcttcagtctgcaagtatggagctcaagttcttaattattcagaatgctgcggttttccaagaggcctttgaaattgttgttcgccatgccaagaactacaccaatgccatgttcaagaacaactacccaagcctgactccacaagcttttgagtttgtgggtgaatttttcacagatgtgtctctctacatcttgggttctgacatcaatgtagatgacatggtcaatgaattgtttgacagcctgtttccagtcatctatacccagctaatgaacccaggcctgcctgattcagccttggacatcaatgagtgcctccgaggagcaagacgtgacctgaaagtatttgggaatttccccaagcttattatgacccaggtttccaagtcactgcaagtcactaggatcttccttcaggctctgaatcttggaattgaagtgatcaacacaactgatcacctgaagttcagtaaggactgtggccgaatgctcaccagaatgtggtactgctcttactgccagggactgatgatggttaaaccctgtggcggttactgcaatgtggtcatgcaaggctgtatggcaggtgtggtggagattgacaagtactggagagaatacattctgtcccttgaagaacttgtgaatggcatgtacagaatctatgacatggagaacgtactgcttggtctcttttcaacaatccatgattctatccagtatgtccagaagaatgcaggaaagctgaccaccactattggcaagttatgtgcccattctcaacaacgccaatatagatctgcttattatcctgaagatctctttattgacaagaaagtattaaaagttgctcatgtagaacatgaagaaaccttatccagccgaagaagggaactaattcagaagttgaagtctttcatcagcttctatagtgctttgcctggctacatctgcagccatagccctgtggcggaaaacgacaccctttgctggaatggacaagaactcgtggagagatacagccaaaaggcagcaaggaatggaatgaaaaaccagttcaatctccatgagctgaaaatgaagggccctgagccagtggtcagtcaaattattgacaaactgaagcacattaaccagctcctgagaaccatgtctatgcccaaaggtagagttctggataaaaacctggatgaggaagggtttgaaagtggagactgcggtgatgatgaagatgagtgcattggaggctctggtgatggaatgataaaagtgaagaatcagctccgcttccttgcagaactggcctatgatctggatgtggatgatgcgcctggaaacagtcagcaggcaactccgaaggacaacgagataagcacctttcacaacctcgggaacgttcattccccgctgaagcttctcaccagcatggccatctcggtggtgtgcttcttcttcctggtgcactgactgcctggtgcccagcacatgtgctgccctacagcaccctgtggtcttcctcgataaagggaaccactttcttatttttttctatttttttttttttgttatcctgtatacctcctccagccatgaagtagaggactaaccatgtgttatgttttcgaaaatcaaatggtatcttttggaggaagatacattttagtggtagcatatagattgtccttttgcaaagaaagaaaaaaaaccatcaagttgtgccaaattattctcctatgtttggctgctagaacatggttaccatgtctttctctctcactccctccctttctatcgttctctctttgcatggatttctttgaaaaaaaataaattgctcaaataaaaaaaaaaaaaaa

SEQ ID NO: 5 - DNA, 2566 bp, Macaca fascicularis
gtagagcggcggcgaacgggcagcttggctcggctgccgggagccaccgcgcgcgctccgcaccctcctctcgcactgtctccgcccggtccccgcacgcggtgccctagtggcccccgccgccctccacgccgcgcccccgcaccccgcaggctaccggctgcacaaccgccgccgccccctggccgcgcggctcgcctcgccccgccccgtctctcctcgctccgccccaccccagtcagccccgccctgccccgcgccgccaagcggttcccgccctcgcccagcgcccaggtagctgcgaggaaacttttgcagcggctgggtagcagcacgtctcttgctccacagggccactgccaggcttgccgagtcctgggactgctctcgctccggctgccactctcctgcgctctcctagctccctgcgaagcaggatggccgggaccgtgcgcaccgcgtgcttggtggtggcgatgctgctcagcttggacttccccggacaggcgcagcccccgccgccgccgccggacgccacctgtcaccaagtccgctccttcttccagagactgcagcccggactcaagtgggtgcccgaaactcccgtgccaggatcagatttgcaagtatgtctccctaagggcccaacatgctgctcaagaaagatggaagaaaaataccaactaacagcacgattgaacatggaacagctgcttcagtctgcaagtatggagctcaagttcttaattattcagaatgctgcagttttccaagaggcctttgaaattgttgttcgccatgccaagaactacaccaatgccatgttcaagaacaactacccaagcctgactccacaagcttttgagtttgtgggtgaatttttcacagatgtgtctctctatatcttgggttctgacatcaatgtggatgacatggtcaatgaattgtttgatagcctgtttccagtcatctatacccaactaatgaacccaggtctgcctgattcagccttggacatcaatgagtgcctccgaggagcaagacgtgacctgaaagtatttgggaacttccccaagcttattatgacccaggtttctaagtcactgcaagtcactaggatcttccttcaggctctgaatcttggaattgaagtgatcaacacaaccgatcacctgaagttcagtaaggactgtggccgaatgctcaccagaatgtggtactgctcttactgccagggactgatgatggttaaaccttgtggtggttactgcaatgtggtcatgcaaggctgtatggcaggtgtggtggagattgacaagtactggagagaatacattctgtctcttgaagagcttgtgaatggcatgtacagaatctatgacatggaaaacgtactgcttggtctcttttcaacaatccacgattctatccagtatgtccagaagaatgcaggaaagctgaccaccactattggcaagttatgtgcccattctcaacaacgccaatatagatctgcttattatcctgaagatctgtttattgacaagaaagtattaaaagttgctcatgtagaacatgaagaaaccttatccagccgaagaagggaactaattcagaagttgaagtctttcatcagcttctatagtgctttgcctggctacatctgcagccatagccctgtggcggaaaacgacaccctttgctggaatggacaagaactcgtggagagatacagccaaaaggcggcaaggaatggaatgaaaaaccagttcaatctccatgagctgaaaatgaagggccctgagccagtagtcagtcaaattattgacaaattgaagcacattaaccagctcctgagaaccatgtctgtgcccaaaggtagagttctggataaaaacctggatgaggaagggtttgaaagtggagactgtggtgatgatgaagatgagtgcattggaggctctggtgatggaatgatgaaagtgaagaatcagctccgcttccttgcagaactggcctatgatctggatgtggatgatgtgcctggaaacaatcagcaggcgactccgaaggacaatgagataagcacctttcacaaccttgggaacgttcattccccgctgaagcttctcaccagcatggccatctcagtggtgtgcttcttcttcctggtgcactgactgcctggtgcccagcacatgtgctgccctacagcaccctgtggtcttcctcgataaagggaaccactttcttatttttttcttttttttttttttatcctgtatacctcctccagccattaagtagaagactaaccatgtgttatgtttttgaaaatcaaatggtatcttttggaggaagataaattttagtggtagtatatagattgtccttttgcaaagaaaagaaaaccatcaagttgtgccaaattattttcctatgtttggctgctagaacatggttaccatgtctttctctctgtcttactccctccctttctatctttctttctctctctctttgcatggatttctttgaaaaaaaaaataaattgctcaaataaaaa

SEQ ID NO: 6 - DNA, 2272 bp, Mus musculus
tgttcccgccctcgcccagcgcccaggtagctgcgaggaaacttttgcggcggctgggtagcggctcctctcttgctctgtcgggctactgccagacttgctgagtctcgggaccgctccggctcttattgccactctctcgtgctctcctcgctcccccaagaagcaggatggccgggaccgtgcgcaccgcgtgcttgctggtggcgatgctgctaggcttgggctgcctgggacaggcgcagcccccgccgcctccagacgccacctgtcaccaggtccgttctttcttccagagactgcagcccggactcaaatgggttccagaaacccctgtaccaggatcagatttgcaagtatgtctccccaagggcccaacatgctgctcaagaaagatggaagaaaaataccaactaacagcacggctgaacatggaacaactgctccagtctgcgagtatggaactcaagttcttaattattcagaatgctgcggttttccaagaggcctttgaaattgttgttcgccatgccaagaactacaccaacgccatgttcaagaataactaccccagcctgactccacaagcttttgagtttgtcggtgaatttttcacagatgtgtctctctacatcttgggttctgatatcaacgtggatgatatggtcaatgaattgttcgacagcctctttccagtcatctacacccagatgatgaacccaggcctgcctgagtcagtcttagacatcaacgagtgcctccgaggagcaagacgtgacctgaaagtatttggcagtttccccaagcttattatgacccaggtttccaagtcactgcaagtcactcgaatcttccttcaagccctgaatctcggaattgaagtcatcaacactaccgaccacctcaagtttagtaaggactgtggccgtatgctcacccgaatgtggtattgctcttactgccagggactgatgatggttaagccttgcggtggttattgcaatgtggtcatgcaaggctgtatggctggtgtggtggagatcgacaagtactggagagaatacattctgtctcttgaagagctcgtgaatggcatgtacagaatctacgacatggagaatgtgctgctcggcctcttttctaccatccatgattccatccagtatgtgcagaagaacggaggcaagctgaccaccaccattggcaagttgtgtgcccactcccagcaacgccaatatagatctgcttattaccctgaagatctgtttattgacaagaagatattaaaagtcgctcatgtcgaacatgaagaaaccttatccagccgaagaagggaactgattcagaaactgaagtctttcatcaacttctatagcgctttgccgggctacatctgcagccatagccccgtggccgaaaatgataccctgtgctggaacggacaagaacttgtggagagatacagccagaaggcggcaaggaacgggatgaagaatcagtttaacctccatgagctgaaaatgaagggccctgagccggtggttagccagatcattgacaaactgaagcacattaaccagctcctgagaaccatgtctgtgcccaagggtaaagttctggataaaagcctggatgaagaaggacttgaaagtggagactgcggtgatgatgaagatgaatgcattggaagctctggtgacgggatggtgaaagtgaagaatcaactgcgcttccttgcagaactggcctatgatctggatgtggacgatgctccggggaacaagcagcatggaaatcagaaggacaacgagatcaccacctctcacagcgtggggaacatgccgtccccactgaagatcctcatcagtgtggccatctatgtggcgtgcttttttttcctggtgcactgacttgccagcgtccagtgcctgtgctgccctgcagcacctgtggtccctacagaaagggagccaccttcttttttttttctttttttttttttttttatcttttatgcctcctcccaccaccattaagtaggagactaaccgcgtgttatgttttcgaaaatcaaatggtatctttatgaggatggtaaattttagtggtaggatagattgtctttttgcaaagaaaaaaaaaaccttcaagttgtgccaaattattttcttacatttgactgttggaacatggttgtcatgtttccctcttttctctttctctgcatggatttctttgacaaaaaaaaataaataaacattcaaataaaaaa

SEQ ID NO: 7 - DNA, 34 bp, Bacteriophage P1
ataacttcgtatagcatacattatacgaagttat

SEQ ID NO: 8 - DNA, 32 bp, Bacteriophage D6
taactttaaataattggcattatttaaagtta

SEQ ID NO: 9 - DNA, 34 bp, Saccharomyces cerevisiae
gaagttcctattctctagaaagtataggaacttc

SEQ ID NO: 10 - DNA, 1743 bp, Homo sapiens
atggccgggaccgtgcgcaccgcgtgcttggtggtggcgatgctgctcagcttggacttcccgggacaggcgcagcccccgccgccgccgccggacgccacctgtcaccaagtccgctccttcttccagagactgcagcccggactcaagtgggtgccagaaactcccgtgccaggatcagatttgcaagtatgtctccctaagggcccaacatgctgctcaagaaagatggaagaaaaataccaactaacagcacgattgaacatggaacagctgcttcagtctgcaagtatggagctcaagttcttaattattcagaatgctgcggttttccaagaggcctttgaaattgttgttcgccatgccaagaactacaccaatgccatgttcaagaacaactacccaagcctgactccacaagcttttgagtttgtgggtgaatttttcacagatgtgtctctctacatcttgggttctgacatcaatgtagatgacatggtcaatgaattgtttgacagcctgtttccagtcatctatacccagctaatgaacccaggcctgcctgattcagccttggacatcaatgagtgcctccgaggagcaagacgtgacctgaaagtatttgggaatttccccaagcttattatgacccaggtttccaagtcactgcaagtcactaggatcttccttcaggctctgaatcttggaattgaagtgatcaacacaactgatcacctgaagttcagtaaggactgtggccgaatgctcaccagaatgtggtactgctcttactgccagggactgatgatggttaaaccctgtggcggttactgcaatgtggtcatgcaaggctgtatggcaggtgtggtggagattgacaagtactggagagaatacattctgtcccttgaagaacttgtgaatggcatgtacagaatctatgacatggagaacgtactgcttggtctcttttcaacaatccatgattctatccagtatgtccagaagaatgcaggaaagctgaccaccactattggcaagttatgtgcccattctcaacaacgccaatatagatctgcttattatcctgaagatctctttattgacaagaaagtattaaaagttgctcatgtagaacatgaagaaaccttatccagccgaagaagggaactaattcagaagttgaagtctttcatcagcttctatagtgctttgcctggctacatctgcagccatagccctgtggcggaaaacgacaccctttgctggaatggacaagaactcgtggagagatacagccaaaaggcagcaaggaatggaatgaaaaaccagttcaatctccatgagctgaaaatgaagggccctgagccagtggtcagtcaaattattgacaaactgaagcacattaaccagctcctgagaaccatgtctatgcccaaaggtagagttctggataaaaacctggatgaggaagggtttgaaagtggagactgcggtgatgatgaagatgagtgcattggaggctctggtgatggaatgataaaagtgaagaatcagctccgcttccttgcagaactggcctatgatctggatgtggatgatgcgcctggaaacagtcagcaggcaactccgaaggacaacgagataagcacctttcacaacctcgggaacgttcattccccgctgaagcttctcaccagcatggccatctcggtggtgtgcttcttcttcctggtgcactga

SEQ ID NO: 11 - DNA, 40 bp, Artificial Sequence
  an artificially synthesized sequence
ggggcgcgtggtggcggctgcagccgccaccacgcgcccc

SEQ ID NO: 12 - DNA, 122 bp, Unknown
  an artificially synthesized sequence
gcgggactctggggttcgaataaagaccgaccaagcgacgtctgagagctccctggcgaattcggtaccaataaaagagctttattttcatgatctgtgtgttggtttttgtgtgcggcgcg

SEQ ID NO: 13 - DNA, 1513 bp, Escherichia coli
ctaccgggtaggggaggcgcttttcccaaggcagtctggagcatgcgctttagcagccccgctgggcacttggcgctacacaagtggcctctggcctcgcacacattccacatccaccggtaggcgccaaccggctccgttctttggtggccccgtcgcgccaccttctactcctcccctagtcaggaagttcccccccgccccgcagctcgcgtcgtgcaggacgtgacaaatggaagtagcacgtctcactagtctcgtgcagatggacagcaccgctgagcaatggaagcgggtaggcctttggggcagcggccaatagcagctttgctccttcgctttctgggctcagaggctgggaaggggtgggtccgggggcgggctcaggggcgggctcaggggcggggcgggcgcccgaaggtcctccggaggcccggcattctgcacgcttcaaaagcgcacgtctgccgcgctgttctcctcttcctcatctccgggcctttcgacctgcagcagcacgtgttgacaattaatcatcggcatagtatatcggcatagtataatacgacaaggtgaggaactaaaccatgggatcggccattgaacaagatggattgcacgcaggttctccggccgcttgggtggagaggctattcggctatgactgggcacaacagacgatcggctgctctgatgccgccgtgttccggctgtcagcgcaggggcgcccggttctttttgtcaagaccgacctgtccggtgccctgaatgaactgcaggacgaggcagcgcggctatcgtggctggccacgacgggcgttccttgcgcagctgtgctcgacgttgtcactgaagcgggaagggactggctgctattgggcgaagtgccggggcaggatctcctgtcatctcaccttgctcctgccgagaaagtatccatcatggctgatgcaatgcggcggctgcatacgcttgatccggctacctgcccattcgaccaccaagcgaaacatcgcatcgagcgagcacgtactcggatggaagccggtcttgtcgatcaggatgatctggacgaagagcatcaggggctcgcgccagccgaactgttcgccaggctcaaggcgcgcatgcccgacggcgaggatctcgtcgtgacccatggcgatgcctgcttgccgaatatcatggtggaaaatggccgcttttctggattcatcgactgtggccggctgggtgtggcggaccgctatcaggacatagcgttggctacccgtgatattgctgaagagcttggcggcgaatgggctgaccgcttcctcgtgctttacggtatcgccgcccccgattcgcagcgcatcgccttctatcgccttcttgacgagttcttctgagcgggactctggggttcgaataaagaccgaccaagcgacgtctgagagctccctggcgaattcggtaccaataaaagagctttattttcatgatctgtgtgttggtttttgtgtgcggcgcg

SEQ ID NO: 14 - DNA, 20 bp, Mus musculus
tggatcctgagaacttcagg

SEQ ID NO: 15 - DNA, 654 bp, Mus musculus
gtgagtctgatgggcacctcctgggtttccttcccctggctattctgctcaaccttcctatcagaaggaaaggggaagcgattctagggagcagtctccatgactgtgtgtggagtgttgacaagagtttggatattttattctctactcagaatcgctgctccccctcactctgttctgtgttgtcatttcctctttctttggtaagcttttaatttccagttgcattttactaaattaattaagctggttatttacttcccatcctgatatcagcttcccctcctcctttcctcccagtccttctctctctcctctctctttctctaatcctttcctttccctcagttcatttcttcttctttgatctacttttgtttgtctttttaaatattgccttgtaacttactcagaggacaaggaagatatgtccctgtttcttctcatagctctcaagaatagtagcataattggcttttatgccagggtgacaggggaagaatatattttacatataaattctgtttgacataggattcttataataatttgtcagcagtttaaggttgcaaacaaatgtctttataaataagcctgcagtatctggtatttttgctctacagttatgttgatggttcttccatattcccacag

SEQ ID NO: 16 - DNA, 871 bp, Mus musculus
ctcctgggcaatcggaattcgcggccgcgatcgtgattgtgctgggccaccaccttggcaaggatttcacccccgctgcacaggctgccttccagaaggtggtggctggagtggccgctgccctggctcacaagtaccactaaaccccctttcctgctcttgcctgtgaacaatggttaattgttcccaagagagcatctgtcagttgttggcaaaatgataaagacatttgaaaatctgtcttctgacaaataaaaagcatttatttcactgcaatgatgttttaaattatttgtctgtgtcatagaagggtttatgctaagttttcaagatacaaagaagtgagggttcaggtctgaccttggggaaataaatgaattacacttcaaatgtatgggacagcaagcagtaagccacagatcctattgccatgccctaaacactcagagaaaaattcaacaaatggtttcatttatacactacattatgattacattttatgtaaattatttgttttttctactcttccacataaatgtctttttttcctcttacctacccagcacttcacagttctcaagccaataatttttcttttgtaaaattaccattattctctaaacttttccctctgtgtttaccaagcaacattatttatcttttcataaatcctgttgccttagacagctccaatagcaatagaggtatgattaaggagagaatagaagtgccctgtttgtcataccatgcctgcacagtcaatagtcactatgagatttcaaatggcactttgcctgggacctttacacctcacaccatactctggcttgagttaggagttaagaatgagagaaatataagatctgtcgac

SEQ ID NO: 17 - DNA, 359 bp, Mus musculus
cttgccagcgtccagtgcctgtgctgccctgcagcacctgtggtccctacagaaagggagccaccttcttttttttttctttttttttttttttttatcttttatgcctcctcccaccaccattaagtaggagactaaccgcgtgttatgttttcgaaaatcaaatggtatctttatgaggatggtaaattttagtggtaggatagattgtctttttgcaaagaaaaaaaaaaccttcaagttgtgccaaattattttcttacatttgactgttggaacatggttgtcatgtttccctcttttctctttctctgcatggatttctttgacaaaaaaaaataaataaacattcaaataaa

SEQ ID NO: 18 - DNA, 31 bp, Artificial Sequence
  an artificially synthesized sequence
agatggctgcctgtgacatttctggaagtgt

SEQ ID NO: 19 - DNA, 30 bp, Artificial Sequence
  an artificially synthesized sequence
ctgaattagttcccttcttcggctggataa

SEQ ID NO: 20 - DNA, 26 bp, Artificial Sequence
  an artificially synthesized sequence
atgagacccagcaagctacacgggct

SEQ ID NO: 21 - DNA, 24 bp, Artificial Sequence
  an artificially synthesized sequence
acttgagctccatacttgcagact

SEQ ID NO: 22 - DNA, 25 bp, Artificial Sequence
  an artificially synthesized sequence
tgatgatgaagatgagtgcattgga

SEQ ID NO: 23 - DNA, 23 bp, Artificial Sequence
  an artificially synthesized sequence
tggccagaactacgggtccagct

SEQ ID NO: 24 - DNA, 23 bp, Artificial Sequence
  an artificially synthesized sequence
agggccctgagccagtggtcagt

SEQ ID NO: 25 - DNA, 23 bp, Artificial Sequence
  an artificially synthesized sequence
tagcggctcctctcttgctctgt

SEQ ID NO: 26 - DNA, 30 bp, Artificial Sequence
  an artificially synthesized sequence
gcccggggcatgtggacagagtcccatact

SEQ ID NO: 27 - DNA, 21 bp, Artificial Sequence
  an artificially synthesized sequence
gaaaccttatccagccgaaga

SEQ ID NO: 28 - DNA, 19 bp, Artificial Sequence
  an artificially synthesized sequence
gcaaagggtgtcgttttcc

SEQ ID NO: 29 - DNA, 20 bp, Artificial Sequence
  an artificially synthesized sequence
caggtagctgcgaggaaact

SEQ ID NO: 30 - DNA, 20 bp, Artificial Sequence
  an artificially synthesized sequence
ccgacagagcaagagaggag

SEQ ID NO: 31 - protein, 443 aa, Artificial Sequence
  an artificially synthesized sequence
QVQLVQSGAEVKKPGASVKVSCKASGYTFTDYEMHWIRQPPGQGLEWIGAIDPKTGDTAYSQKFKGRVTLTADKSTSTAYMELSSLTSEDTAVYYCTRFYSYTYWGQGTLVTVSSASTKGPSVFPLAPSSKSTSGGTAALGCLVKDYFPEPVTVSWNSGALTSGVHTFPAVLQSSGLYSLSSVVTVPSSSLGTQTYICNVNHKPSNTKVDKKVEPKSCDKTHTCPPCPAPELRGGPKVFLFPPKPKDTLMISRTPEVTCVVVDVSHEDPEVKFNWYVDGVEVHNAKTKPREEQYASTYRVVSVLTVLHQDWLNGKEYKCKVSNKALPAPIEKTISKAKGQPREPQVYTLPPSRDELTKNQVSLTCLVKGFYPSDIAVEWESNGQPENNYKTTPPYLDSDGSFFLYSKLTVDKSRWQQGNVFSCSVMHEALHNHYTQESLSLSP

SEQ ID NO: 32 - protein, 219 aa, Artificial Sequence
  an artificially synthesized sequence
DIVMTQSPLSLPVTPGEPASISCRSSQSLVHSNRNTYLHWYQQKPGQAPRLLIYKVSNRFSGVPDRFSGSGSGTDFTLKISRVEAEDVGVYYCSQNTHVPPTFGQGTKLEIKRTVAAPSVFIFPPSDEQLKSGTASVVCLLNNFYPREAKVQWKVDNALQSGNSQESVTEQDSKDSTYSLSSTLTLSKADYEKHKVYACEVTHQGLSSPVTKSFNRGEC

SEQ ID NO: 33 - protein, 444 aa, Artificial Sequence
  an artificially synthesized sequence
EVQLVESGGGLVQPGKSLKLSCEASGFTFSGYGMHWVRQAPGRGLESVAYITSSSINIKYADAVKGRFTVSRDNAKNLLFLQMNILKSEDTAMYYCARFDWDKNYWGQGTMVTVSSASTKGPSVFPLAPSSKSTSGGTAALGCLVKDYFPEPVTVSWNSGALTSGVHTFPAVLQSSGLYSLSSVVTVPSSSLGTQTYICNVNHKPSNTKVDKKVEPKSCDKTHTCPPCPAPELRGGPKVFLFPPKPKDTLMISRTPEVTCVVVDVSHEDPEVKFNWYVDGVEVHNAKTKPREEQYASTYRVVSVLTVLHQDWLNGKEYKCKVSNKALPAPIEKTISKAKGQPREPQVYTLPPSRKELTKNQVSLTCLVKGFYPSDIAVEWESNGQPENNYKTTPPYLDSDGSFFLYSKLTVDKSRWQQGNVFSCSVMHEALHNHYTQKSLSLSP

SEQ ID NO: 34 - protein, 214 aa, Artificial Sequence
  an artificially synthesized sequence
DIQMTQSPSSLPASLGDRVTINCQASQDISNYLNWYQQKPGKAPKLLIYYTNKLADGVPSRFSGSGSGRDSSFTISSLESEDIGSYYCQQYYNYPWTFGPGTKLEIKRTVAAPSVFIFPPSDEQLKSGTASVVCLLNNFYPREAKVQWKVDNALQSGNSQESVTEQDSKDSTYSLSSTLTLSKADYEKHKVYACEVTHQGLSSPVTKSFNRGEC

SEQ ID NO: 35 - DNA, 20 bp, Artificial Sequence
  an artificially synthesized sequence
tatcagagcttggttgacgg

SEQ ID NO: 36 - DNA, 32 bp, Artificial Sequence
  an artificially synthesized sequence
actcgttgtggcttagaagcagtaacaatacc

SEQ ID NO: 37 - DNA, 30 bp, Artificial Sequence
  an artificially synthesized sequence
actgtaatcctagtacttaggaggctgagg

SEQ ID NO: 38 - DNA, 26 bp, Artificial Sequence
  an artificially synthesized sequence
aatccatcttgttcaatggccgatcc

SEQ ID NO: 39 - DNA, 30 bp, Artificial Sequence
  an artificially synthesized sequence
tagcagccttcagatgaagaggtaggactc

SEQ ID NO: 40 - DNA, 28 bp, Artificial Sequence
  an artificially synthesized sequence
ttgatgtgccacctcactgctgcactgg

SEQ ID NO: 41 - DNA, 24 bp, Artificial Sequence
  an artificially synthesized sequence
aactgacaatgggacatcagctga

SEQ ID NO: 42 - DNA, 24 bp, Artificial Sequence
  an artificially synthesized sequence
atgggactgttactttactaagat

SEQ ID NO: 43 - DNA, 28 bp, Artificial Sequence
  an artificially synthesized sequence
aagaaatgggtggtattacacagacacc

SEQ ID NO: 44 - DNA, 31 bp, Artificial Sequence
  an artificially synthesized sequence
tgggccagcgggaggcagtgttctccagagg

SEQ ID NO: 45 - DNA, 29 bp, Artificial Sequence
  an artificially synthesized sequence
tagttcggtgacctggctttatctactgg

SEQ ID NO: 46 - DNA, 31 bp, Artificial Sequence
  an artificially synthesized sequence
atggctgcttctagaagccaccagtctcagg

SEQ ID NO: 47 - DNA, 26 bp, Artificial Sequence
  an artificially synthesized sequence
tgctccacgcttttgccggaggacag

SEQ ID NO: 48 - DNA, 25 bp, Artificial Sequence
  an artificially synthesized sequence
taggaggagaacacctggactactc

SEQ ID NO: 49 - DNA, 28 bp, Artificial Sequence
  an artificially synthesized sequence
agcattctgagaggatgcggtggaacac

SEQ ID NO: 50 - DNA, 29 bp, Artificial Sequence
  an artificially synthesized sequence
tgctcggagggctggatctgggtccacag

SEQ ID NO: 51 - DNA, 29 bp, Artificial Sequence
  an artificially synthesized sequence
tcatcctgtggcttgcctctatttgttgc

SEQ ID NO: 52 - DNA, 29 bp, Artificial Sequence
  an artificially synthesized sequence
ttgctatggcactttgagaaacctccatc

SEQ ID NO: 53 - DNA, 26 bp, Artificial Sequence
  an artificially synthesized sequence
aatacttctactggagaagcaaagag

SEQ ID NO: 54 - DNA, 27 bp, Artificial Sequence
  an artificially synthesized sequence
tagttgcatttagaggacttattatgc

SEQ ID NO: 55 - DNA, 360 bp, Artificial Sequence
  an artificially synthesized sequence
  CDS (1)..(360)
gaagtgcagctggtcgagagcgggggggggctggtgcagccaggaggatctctgaggctgagttgcgccgcttcaggcttcaacatcaaggacacttacattcactgggtgcgacaggcaccagggaaaggactggagtgggtcgcccggatctatcccacaaatggatacactcggtatgccgactccgtgaagggcagattcaccattagcgccgatacctccaaaaacacagcttacctgcagatgaacagcctgagggctgaagatacagcagtgtactattgctctcgctggggaggcgacggcttttacgcaatggattattggggccaggggactctggtgaccgtcagctcc

SEQ ID NO: 56 - protein, 120 aa, Artificial Sequence [sequence omitted]

SEQ ID NO: 57 - DNA, 321 bp, Artificial Sequence
  an artificially synthesized sequence
  CDS (1)..(321)
gacattcagatgactcagagcccttcaagcctgagtgcttcagtcggggacagggtgacaatcacttgccgcgcaagccaggatgtcaacaccgctgtggcatggtaccagcagaagccaggcaaagcacccaagctgctgatctacagcgcctccttcctgtattccggggtgccatctcggttttctggcagtagatcagggaccgacttcaccctgacaatcagctccctgcagcccgaagattttgccacatactattgccagcagcactacaccacaccccctacattcgggcagggaactaaagtggagattaag

SEQ ID NO: 58 - protein, 107 aa, Artificial Sequence [sequence omitted]

SEQ ID NO: 59 - DNA, 321 bp, Artificial Sequence
  an artificially synthesized sequence
  CDS (1)..(321)
gatattcagatgactcagagcccttcttcactgagtgcatcagtgggcgaccgagtcaccatcacatgccgggccagccaggatattagaaactacctgaattggtatcagcagaagcctggcaaagctccaaagctgctgatctactatacctctaggctggagagtggagtgccatcacgcttcagcggatccggatctgggaccgactacactctgaccattagctccctgcagccagaagatttcgccacatactattgtcagcagggaaacactctgccctggacctttggacagggcaccaaagtggagatcaag

SEQ ID NO: 60 - protein, 107 aa, Artificial Sequence [sequence omitted]

SEQ ID NO: 61 - DNA, 366 bp, Artificial Sequence
  an artificially synthesized sequence
  CDS (1)..(366)
gaggtgcagctggtcgaatccggaggaggactggtgcagccaggaggaagcctgcgactgtcctgcgccgctagcggatactcctttacaggctatactatgaattgggtgcgacaggctcccgggaaaggactggagtgggtggcactgatcaacccttacaagggcgtcagtacctataatcagaagttcaaagaccggttcaccatttctgtggataagagtaaaaacaccgcttacctgcagatgaatagcctgagagcagaggacacagccgtgtactattgcgcaaggagtggctactatggggactcagattggtatttcgacgtgtggggacaggggaccctggtgacagtctctagt

SEQ ID NO: 62 - protein, 122 aa, Artificial Sequence [sequence omitted]

SEQ ID NO: 63 - protein, 118 aa, Artificial Sequence
  an artificially synthesized sequence
QVQLVESGGGVVQPGRSLRLSCAASGFTFSSYTMHWVRQAPGKGLEWVTFISYDGNNKYYADSVKGRFTISRDNSKNTLYLQMNSLRAEDTAIYYCARTGWLGPFDYWGQGTLVTVSS

SEQ ID NO: 64 - protein, 108 aa, Artificial Sequence
  an artificially synthesized sequence
EIVLTQSPGTLSLSPGERATLSCRASQSVGSSYLAWYQQKPGQAPRLLIYGAFSRATGIPDRFSGSGSGTDFTLTISRLEPEDFAVYYCQQYGSSPWTFGQGTKVEIK

SEQ ID NO: 65 - protein, 324 aa, Artificial Sequence
  an artificially synthesized sequence
AKTTPPSVYPLAPGSAAQTNSMVTLGCLVKGYFPEPVTVTWNSGSLSSGVHTFPAVLQSDLYTLSSSVTVPSSTWPSETVTCNVAHPASSTKVDKKIVPRDCGCKPCICTVKEVSKVFIFPPKPKDVLTITLTPKVTCVVVDISKDDPEVQFSWFVDDVEVHTAQTQPREEQFNSTFRSVSELPIMHQDWLNGKEFKCRVNSAAFPAPIEKTISKTKGRPKAPQVYTIPPPKEQMAKDKVSLTCMITDFFPEDITVEWQWNGQPAENYKNTQPIMDTDGSYFVYSELNVQKSNWEAGNTFTCSVLHEGLHNHHTEKSLSHSPGK

SEQ ID NO: 66 - protein, 107 aa, Artificial Sequence
  an artificially synthesized sequence
RADAAPTVSIFPPSSEQLTSGGASVVCFLNNFYPKDINVKWKIDGSERQNGVLNSWTDQDSKDSTYSMSSTLTLTKDEYERHNSYTCEATHKTSTSPIVKSFNRNEC

SEQ ID NO: 67 - protein, 122 aa, Artificial Sequence
  an artificially synthesized sequence
QVQLVESGGGVVQPGGSLRLSCAASGFTFSNAWMHWVRQAPGKGLEWVAQIKDKSQNYATYVAESVKGRFTISRADSKNSIYLQMNSLKTEDTAVYYCRYVHYAAGYGVDIWGQGTTVTVSS

SEQ ID NO: 68 - protein, 112 aa, Artificial Sequence
  an artificially synthesized sequence
DIVMTQSPLSLPVTPGEPASISCRSSQPLVHSNRNTYLHWYQQKPGQAPRLLIYKVSNRFSGVPDRFSGSGSGTDFTLKISRVEAEDVGVYYCGQGTQVPYTFGQGTKLEIK

SEQ ID NO: 69 - protein, 324 aa, Artificial Sequence
  an artificially synthesized sequence
AKTTPPSVYPLAPGSAAQTNSMVTLGCLVKGYFPEPVTVTWNSGSLSSGVHTFPAVLQSDLYTLSSSVTVPSSTWPSETVTCNVAHPASSTKVDKKIVPRDCGCKPCICTVKEVSKVFIFPPKPKDVLTITLTPKVTCVVVDISKDDPEVQFSWFVDDVEVHTAQTQPREEQFNSTFRSVSELPIMHQDWLNGKEFKCRVNSAAFPAPIEKTISKTKGRPKAPQVYTIPPPKEQMAKDKVSLTCMITDFFPEDITVEWQWNGQPAENYKNTQPIMRTDGSYFVYSKLNVQKSNWEAGNTFTCSVLHEGLHNHHTEKSLSHSPGK

SEQ ID NO: 70 - protein, 325 aa, Artificial Sequence
  An artificially generated sequence
ASTKGPSVFPLAPCSRSTSESTAALGCLVKDYFPEPVTVSWNSGALTSGVHTFPAVLQSSGLYSLSSVVTVPSSSLGTKTYTCNVDHKPSNTKVDKRVESKYGPPCPPCPAPEFRGGPKVFLFPPKPKDTLMISRTPEVTCVVVDVSQEDPEVQFNWYVDGVEVHNAKTKPREEQFASTYRVVSVLTVLHQDWLNGKEYKCKVSNKGLPSSIEKTISKAKGQPREPQVYTLPPSQKEMTKNQVSLTCLVKGFYPSDIAVEWESNGQPENNYKTTPPVLDSDGSFFLYSKLTVDKSRWQEGNVFSCSVMHEALHNHYTQKSLSLSP

SEQ ID NO: 71 - protein, 115 aa, Artificial Sequence
  An artificially generated sequence
QVQLVQSGAEVKKPGASVTVSCKASGYTFTDYEMHWIRQPPGEGLEWIGAIDGPTPDTAYSEKFKGRVTLTADKSTSTAYMELSSLTSEDTAVYYCTRFYSYTYWGQGTLVTVSS

SEQ ID NO: 72 - protein, 325 aa, Artificial Sequence
  An artificially generated sequence
ASTKGPSVFPLAPCSRSTSESTAALGCLVKDYFPEPVTVSWNSGALTSGVHTFPAVLQSSGLYSLSSVVTVPSSSLGTQTYTCNVDHKPSNTKVDKRVESKYGPPCPPCPAPEFRGGPKVFLFPPKPKDTLMISRTPEVTCVVVDVSQEDPEVQFNWYVDGVEVHNAKTKPREEQFASTYRVVSVLTVLHQDWLNGKEYKCKVSNKGLPSSIEKTISKAKGQPREPQVYTLPPSQEEMTKNQVSLTCLVKGFYPSDIAVEWESNGQPENNYKTTPPVLDSDGSFFLYSKLTVDKSRWQEGNVFSCSVMHEALHNHYTQESLSLSP

SEQ ID NO: 73 - protein, 112 aa, Artificial Sequence; identical to SEQ ID NO: 68
  An artificially generated sequence

SEQ ID NO: 74 - protein, 107 aa, Artificial Sequence [sequence omitted]